European Patent Specification EP 3 768 237 B1, published May 15, 2024. Title: LIVER PROTECTANT COMPOSITIONS AND THERAPEUTIC APPLICATIONS. Applicant: Majeed, Muhammed Nagabhushanam, Kalyanam Mundkur, Lakshmi. The sequence listing filed with the application follows.

SEQUENCE LISTING (12 sequences)

SEQ ID NO: 1 - DNA, 20 bp, Artificial Sequence
  Forward primer for beta-actin
gaagtccctcaccctcccaa

SEQ ID NO: 2 - DNA, 16 bp, Artificial Sequence
  Reverse Primer for beta-actin
ggcatggacgcgacca

SEQ ID NO: 3 - DNA, 24 bp, Artificial sequence
  Forward primer for NFkappaB
gaaattcctgatccagacaaaaac

SEQ ID NO: 4 - DNA, 24 bp, Artificial sequence
  Reverse primer for NFkappaB
atcacttcaatggcctctgtgtag

SEQ ID NO: 5 - DNA, 19 bp, Artificial sequence
  Forward primer for TNF-alpha
ctccaggcggtgcctatgt

SEQ ID NO: 6 - DNA, 17 bp, Artificial sequence
  Reverse primer for TNF-alpha
gaagagcgtggtggccc

SEQ ID NO: 7 - DNA, 19 bp, Artificial sequence
  Forward primer for MCP-1
gcatccacgtgttggctca

SEQ ID NO: 8 - DNA, 23 bp, Artificial sequence
  Reverse primer for MCP-1
ctccagcctactcattgggatca

SEQ ID NO: 9 - DNA, 22 bp, Artificial sequence
  Forward primer for TGF-beta
ttgccctctacaaccaacacaa

SEQ ID NO: 10 - DNA, 20 bp, Artificial sequence
  Reverse primer for TGF-beta
ggcttgcgacccacgtagta

SEQ ID NO: 11 - DNA, 21 bp, Artificial sequence
  Forward primer for Collagen1
ttccctggacctaagggtact

SEQ ID NO: 12 - DNA, 18 bp, Artificial sequence
  Reverse primer for Collagen1
ttgagctccagcttcgcc